European Patent Specification EP 3 331 542 B1, published July 1, 2026. Title: COMPOSITIONS AND METHODS FOR TREATING CANCERS. Applicant: ENB Therapeutics Jamal, Sumayah. Application PCT/US16/45343. The sequence listing filed with the application follows.

SEQUENCE LISTING (1 sequence)

SEQ ID NO: 1 - protein, 20 aa, Artificial Sequence
  Synthetic
  MISC_FEATURE (1)..(1): Acetylation
  MISC_FEATURE (20)..(20): Carboxylation
AAVALLPAVLLAALAPIETD